European Patent Specification EP 3 675 875 B1, published December 11, 2024. Title: CORE-SHELL PARTICLES COMPRISING METAL OXIDE AND LANTHANIDE ELEMENT. Applicant: Bar Ilan University. The sequence listing filed with the application follows.

SEQUENCE LISTING (4 sequences)

SEQ ID NO: 1 - DNA, 20 bp, Mus musculus
ctggatgccgcaaacatgtc

SEQ ID NO: 2 - DNA, 19 bp, Mus musculus
ctgccgctgtgacccactc

SEQ ID NO: 3 - DNA, 23 bp, Leishmania donovani
agtacggctgcgacaccttggag

SEQ ID NO: 4 - DNA, 22 bp, Leishmania donovani
gttccggccccacggcatcacc